European Patent Specification EP 4 404 988 B1, published October 29, 2025. Title: Non-adhesive collagen-like hydrogels. Applicant: Evonik Operations GmbH. The sequence listing filed with the application follows.

SEQUENCE LISTING (9 sequences)

SEQ ID NO: 1 - protein, 330 aa, Streptococcus pyogenes
NHKVHMHHHHHHADEQEEKAKVRTELIQELAQGLGGIEKKNFPTLGDEDLDHTYMTKLLTYLQEREQAENSWRKRLLKGIQDHALDLVPRGSPGLPGPRGEQGPTGPTGPAGPRGLQGLQGLQGERGEQGPTGPAGPRGLQGERGEQGPTGLAGKAGEAGAKGETGPAGPQGPRGEQGPQGLPGKDGEAGAQGPAGPMGPAGERGEKGEPGTQGAKGDRGETGPVGPRGERGEAGPAGKDGERGPVGPAGKDGQNGQDGLPGKDGKDGQNGKDGLPGKDGKDGQNGKDGLPGKDGKDGQDGKDGLPGKDGKDGLPGKDGKDGQPGKPGKY

SEQ ID NO: 2 - protein, 292 aa, Streptococcus pyogenes
NHKVHMHHHHHHDHTYMTKLLTYLQEREQAENSWRKRLLKGIQDHALDLVPRGSPGLPGPRGEQGPTGPTGPAGPRGLQGLQGLQGERGEQGPTGPAGPRGLQGERGEQGPTGLAGKAGEAGAKGETGPAGPQGPRGEQGPQGLPGKDGEAGAQGPAGPMGPAGERGEKGEPGTQGAKGDRGETGPVGPRGERGEAGPAGKDGERGPVGPAGKDGQNGQDGLPGKDGKDGQNGKDGLPGKDGKDGQNGKDGLPGKDGKDGQDGKDGLPGKDGKDGLPGKDGKDGQPGKPGKY

SEQ ID NO: 3 - protein, 267 aa, Streptococcus pyogenes
NHKVHMHHHHHHLLKGIQDHALDLVPRGSPGLPGPRGEQGPTGPTGPAGPRGLQGLQGLQGERGEQGPTGPAGPRGLQGERGEQGPTGLAGKAGEAGAKGETGPAGPQGPRGEQGPQGLPGKDGEAGAQGPAGPMGPAGERGEKGEPGTQGAKGDRGETGPVGPRGERGEAGPAGKDGERGPVGPAGKDGQNGQDGLPGKDGKDGQNGKDGLPGKDGKDGQNGKDGLPGKDGKDGQDGKDGLPGKDGKDGLPGKDGKDGQPGKPGKY

SEQ ID NO: 4 - protein, 240 aa, Streptococcus pyogenes
GSPGLPGPRGEQGPTGPTGPAGPRGLQGLQGLQGERGEQGPTGPAGPRGLQGERGEQGPTGLAGKAGEAGAKGETGPAGPQGPRGEQGPQGLPGKDGEAGAQGPAGPMGPAGERGEKGEPGTQGAKGDRGETGPVGPRGERGEAGPAGKDGERGPVGPAGKDGQNGQDGLPGKDGKDGQNGKDGLPGKDGKDGQNGKDGLPGKDGKDGQDGKDGLPGKDGKDGLPGKDGKDGQPGKPGKY

SEQ ID NO: 5 - protein, 267 aa, Streptococcus pyogenes
NHKVHMHHHHHHLLKGIQDHALDLVPRGSPGLPGPRGEQGPTGPTGPAGPRGLQGLQGLQGERGEQGPTGPAGPRGLQGERGEQGPTGLAGKAGEAGAKGETGPAGPQGPRGEQGPQGLPGKDGEAGAQGPAGPMGPAGERGEKGEPGTQGAKGDRGETGPAGPRGERGEAGPAGKDGERGPVGPAGKDGQNGQDGLPGKDGKDGQNGKDGLPGKDGKDGQNGKDGLPGKDGKDGQDGKDGLPGKDGKDGLPGKDGKDGQPGKPGKY

SEQ ID NO: 6 - protein, 267 aa, Streptococcus pyogenes
NHKVHMHHHHHHLLKGIQDHALDLVPRGSPGLPGPRGEQGPTGPTGPAGPRGLQGLQGLQGERGEQGPTGPAGPRGLQGERGEQGPTGLAGKAGEAGAKGETGPAGPQGPRGEQGPQGLPGKDGEAGAQGPAGPMGPAGERGEKGEPGTQGAKGDRGETGPQGPRGERGEAGPAGKDGERGPVGPAGKDGQNGQDGLPGKDGKDGQNGKDGLPGKDGKDGQNGKDGLPGKDGKDGQDGKDGLPGKDGKDGLPGKDGKDGQPGKPGKY

SEQ ID NO: 7 - protein, 267 aa, Streptococcus pyogenes
NHKVHMHHHHHHLLKGIQDHALDLVPRGSPGLPGPRGEQGPTGPTGPAGPRGLQGLQGLQGERGEQGPTGPAGPRGLQGERGEQGPTGLAGKAGEAGAKGETGPAGPQGPRGEQGPQGLPGKDGEAGAQGPAGPMGPAGERGEKGEPGTQGAKGDRGETGPVGPAGERGEAGPAGKDGERGPVGPAGKDGQNGQDGLPGKDGKDGQNGKDGLPGKDGKDGQNGKDGLPGKDGKDGQDGKDGLPGKDGKDGLPGKDGKDGQPGKPGKY

SEQ ID NO: 8 - protein, 267 aa, Streptococcus pyogenes
NHKVHMHHHHHHLLKGIQDHALDLVPRGSPGLPGPRGEQGPTGPTGPAGPRGLQGLQGLQGERGEQGPTGPAGPRGLQGERGEQGPTGLAGKAGEAGAKGETGPAGPQGPRGEQGPQGLPGKDGEAGAQGPAGPMGPAGERGEKGEPGTQGAKGDRGETGPSGPRGERGEAGPAGKDGERGPVGPAGKDGQNGQDGLPGKDGKDGQNGKDGLPGKDGKDGQNGKDGLPGKDGKDGQDGKDGLPGKDGKDGLPGKDGKDGQPGKPGKY

SEQ ID NO: 9 - protein, 267 aa, Streptococcus pyogenes
NHKVHMHHHHHHLLKGIQDHALDLVPRGSPGLPGPRGEQGPTGPTGPAGPRGLQGLQGLQGERGEQGPTGPAGPRGLQGERGEQGPTGLAGKAGEAGAKGETGPAGPQGPRGEQGPQGLPGKDGEAGAQGPAGPMGPAGERGEKGEPGTQGAKGDRGETGPVGPKGERGEAGPAGKDGERGPVGPAGKDGQNGQDGLPGKDGKDGQNGKDGLPGKDGKDGQNGKDGLPGKDGKDGQDGKDGLPGKDGKDGLPGKDGKDGQPGKPGKY